European Patent Application EP 4 151 727 A1, published March 22, 2023. Title: Neue Urethanasen fuer den Abbau von Polyurethanen. Applicant: Covestro Deutschland AG. The sequence listing filed with the application follows.

SEQUENCE LISTING (12 sequences)

SEQ ID NO: 1 - protein, 469 aa, unidentified
  REGION 1..469: note = Derived from metagenome
MMGGVGVREELATWTAVRLAEHIRKKELSPVEVTDYFLRRIEALNPAVNAFCTVDADGAMRAAKAAEQRLMAGETPPLLGVPVAIKDLTPTKGIRTTYGSRLFADNVPEADAVLVTRLKQAGAIIVGKTNTPEFGHAGVTDNRLFGRTNNPWDLSRIAGGSSGGSDGGGSIRIPASCCGIFGFKPTFGRVPHDTGATAFSITAPFLHHGPMSRTVEDSVLMLAAMQGPDGCDPFSLPLPGIDWPLSAEIKPFSQWRIAYSPNLDFYAIDPAVRQVMEQAVSALQGLGCRVEEVRLGLEEGKTLVLETFARLWAVHYAAFYEELLEREAELSKGFVATIRYGQQFSAVEYKRLERPRAVVYERVENVFAKYDLLITPTLAVPPFAHDCPPREIDGKAVNPYNEWMLTSIFNLTGHPVASIPAGFSPEGLPIGMQIVGPRLADAAVLEFAYLFEQTVAPRRPYPCDDVRLN

SEQ ID NO: 2 - protein, 264 aa, unidentified
  REGION 1..264: note = Derived from metagenome
  SITE 252: note = misc_feature - Xaa can be any naturally occurring amino acid
LDYLGGFSPLESDVTVEKTRIAGVPGEWISTPDARKDRVLFYLHGGAYCFGSCDSHRGLVSRLARACGSRALLIEYRLAPEHPFPAALEDSTAAYRELIRSGVRPENLVIAGDSAGGGLTMATLLTLRDEGDPLPSAAVLLSPWTDLEGTGESMKTKADVEPWLDPEKSHLLAKLYLGDLDPRHPLVSPIHADLNNLPPLLVHVGSDECLLDDSVRLVERAKSAGVETEFKICDEMWHVFHGFPIPEAQQAXEEIGAFVRARLP

SEQ ID NO: 3 - protein, 297 aa, unidentified
  REGION 1..297: note = Derived from metagenome
MASPQSEAIRQMLREQKEAAKKGAPSIEEQRRQLDYLGGFSPLESDVTVEKTRIAGVPGEWISTPDARKDRVLFYLHGGAYCFGSCDSHRGLVSRLARACGSRALLIEYRLAPEHPFPAALEDSTAAYRELIRSGVRPENLVIAGDSAGGGLTMATLLTLRDEGDPLPSAAVLLSPWTDLEGTGESMKTKADVEPWLDPEKSHLLAKLYLGDLDPRHPLVSPIHADLNNLPPLLVHVGSDECLLDDSVRLVERAKSAGVETEFKIWDEMWHVFHGFPIPEAQQAIEEIGAFVRARLP

SEQ ID NO: 4 - protein, 311 aa, unidentified
  REGION 1..311: note = Derived from metagenome
MADPQLEAVLVGLAQASAGAQGPATVEGFRVALRELTRMLDFRDIPVGRVENRMIPGPDGEIGIRIYTPIAAGARMLETLIYFHGGGFVAGDLETHDTLCRGLTARSGCRVISVDYRLAPEHPFPAAIDDSYAALRWIEANATTLGVDSNRIAVGGDSAGGNIAAVVAQLARGAGNPVVRFQLLIYPVVQWDVATPSRQQFAEDPIIPRDVIDMCARNYFGPMVPATDFRAAPLAASDLAGLPPAYVITAGLDPLRDEGAQYAEKLREAGVAVEHVGYDDMIHGFMSMSNALDTAKLAIERAGDALRNALR

SEQ ID NO: 5 - protein, 316 aa, unidentified
  REGION 1..316: note = Derived from metagenome
MSLDPKARELLAMVYRVNAPRFHELSVSQARHATQKLMFAFRPEAPAVASTTEVPIPRPDGSVLFARLYRPLGCHASEDLGLLIYFHGGGWCTGDLPGYDVLCRELANQSGAAVLSVDYRLAPEHRFPAAVHDASLAFEWSTENASLLGVDAERIALGGDSAGGNLAIVAALEARDRAARMPRALALIYPSTQIHSERSSRETFADGYFLDRESLRWFYEHYFADPAQAQSWQASPMLAASLAGLPPAILITAGCDPLTDDCVAFAERMVADGGLVVRHHFEGMVHGFLPLGKFFAQANEAVRCVSSYLREALQAS

SEQ ID NO: 6 - protein, 297 aa, unidentified
  REGION 1..297: note = Derived from metagenome
  SITE 216: note = misc_feature - Xaa can be any naturally occurring amino acid
MSLEELAVVRQLLAGLVTGEARSLEDFRTSYDEAGKAFGLPEGVTVTPVSAGGVPGEWLAPAAGAGKRVLLYLHGGGYALGSLDSHRHLAAHTALALNGRVLLIDYRRSPEHPFPAAVDDALAAYRWLTETGVDPAKLAVAGDSAGGGLTVAVLLAARDAGLRLPAAAVCISPWANLENKGASYGAKANVDPMVRHADLELWTAAYLGTSTPRRAXLASPVYADLNGLPPFLIQVGSSEVLLSDSHLLADRLKEAGVSVDLHVWPEMIHVWHWFAPVLSEGRAAIDEMASFLDTKLG

SEQ ID NO: 7 - protein, 490 aa, unidentified
  REGION 1..490: note = Derived from metagenome
MTGLHFRSASELGRMIRRGEISSAELTDHFIQRIETLDGKTNAVVARDFDRARALAKEADAAQARGASLGALHGLPFTIKDAYEVEGIVSTGGNPTWKDHVPTSSATAVERLQRSGAIVMGKTNVPYLSGDLQTYNDIYGTTNNPWALDCGPGGSSGGSAASLAAGFAAAEFGSDIGGSIRTPAHLCGVFGHKPSFGIVPKRGHLSPPPGCLSEGDLSVAGPLARSAEDLKLLLSLTAGPDWADAAGWKLDLPPARARTPRELRAAVWIDDEFCDIDRESADLLRNAAKALQDAGANVDWNARPDFTLAEITECYLILLHSQIGAGMPQSIRDHWAEMKKGFAPDDKSHAALQAIGGTLSLAERAVWKEVQAQLRWKWHTFFKSYDVVLSPVLMRPAFEHNHQSNWHKRELDVNGVKRPYMDVLIWAGPAVVSYLPATAAPVGVTSEGKPVGIQIIGPHLEDYTTIAVAGMFEEILGGFKPPKGWAAALE

SEQ ID NO: 8 - protein, 177 aa, unidentified
  REGION 1..177: note = Derived from metagenome
CACCLSLVDRDGRRPGELAVAGDSAGGGLTVAVLLAARDAGLRLPAAAVCISPWANLENKGASYGAKANVDPMVRHADLELWTAAYLGTSTPRRAPLASPVYADLNGLPPFLIQVGSSEVLLSDSHLLADRLKEAGVSVDLHVWPEMIHVWHWFAPVLSEGRAAIDEMASFLDTKLG

SEQ ID NO: 9 - protein, 491 aa, unidentified
  REGION 1..491: note = Derived from metagenome
LERSDLDYASATEIARLVRTRQISAADVTEHAISRIEARNGSLNAFVYTDFEQARSRAKDLDTRISAGEDVGPLAGVPTAIKDLFNFYPGWPSTLGGIRCLRDFKLDVKSRYATKMEEAGAVVLGITNSPVLGFRGTTDNDLYGPTRNPFDLSRNSGGSSGGTSAAVADGLLPIGDGTDGGGSIRIPAAWCHVFGFQASPGRIPLAIRPNAFGAAAPFIYEGPITRTVEDAALAMSVLAGSDPADPFSLNDRLDWLGAVDQPITSLRIGFTPDFGGFPVEPAVAATIAHAVRAFEQAGAKIVPLKLDFGYTHDELSQLWCRMISQGTIAVVDSFAENGLHLEPDFPAPVMEWAQKAKNATPLDLHRDQVMRTKVYDVLNAAFSQVDLIAGPTTTCLPTPNGERGMTVGPSEIAGTPINRLIGFCPTFLTNFTGNPAASLPAGLADGLPVGLMLIGPRRDDLTVLSASAAFERVQPWADSYRIPAARPLGSQ

SEQ ID NO: 10 - protein, 330 aa, unidentified
  REGION 1..330: note = Derived from metagenome
MRPRSRPHARARGAPTILRDPATMALHRTPRRNDMADRGIEVVHAHLAKLPPADSLTVAERRAQYERAEKVFPLSPDVKVERVTAGAAPAEWLRPPSARAGHVVLYLHGGGYVIGSPRSHRHLAAAIAGAAGTNALLLDYRLAPEHPFPAALDDAVAAYRWLLDQGIAAEHIAVAGDSAGGGLTVATLLALRDAHLPRPAAGVCISPWVDLTCSGGSYQSKAGVDPIVRQAGVAEMARAYLGATDPRSPLASPLFADLRGLPPLLIHVGSDEVLLDDAIGLAERAKAAGVDATLEQWDRMIHVWHWFLPMLDEAQTAVESIGRFVRARTA

SEQ ID NO: 11 - protein, 544 aa, unidentified
GQPASPPVVDTAQGRVLGKYVSLEGLAQPVAVFLGVPFAKPPLGSLRFAPPQPAEPWSFVKNTTSYPPMCCQDPVAGQMTSDLFTNRKERLIPEFSEDCLYLNIYTPADLTKRGRLPVMVWIHGGGLVVGGASTYDGLALAAHENVVVVAIQYRLGIWGFFSTGDEHSRGNWGHLDQVAALHWVQENIANFGGDPGSVTIFGESAGGESVSVLVLSPLAKNLFHRAISESGVAFTAGLVRKDMKAAAKQIAVLAGCKTTTSAVFVHCLRQKSEDELLDLTLKMKFFALDLHGDPRESHPFLTTVVDGVLLPKMPEEILAEKDFNTVPYIVGINKQEFGWLLPTMMGFPLSEGKLDQKTATSLLWKSYPIANIPEELTPVATDKYLGGTDDPVKKKDLFLDLMGDVVFGVPSVTVARQHRDAGAPTYMYEFQYRPSFSSDKKPKTVIGDHGDEIFSVFGAPFLRGDAPEEEVSLSKTVMKFWANFARSGNPNGEGLPHWPMYDQEEGYLQIGVNTQAAKRLKGEEVAFWNDLLSKEAAKKPPKIK

SEQ ID NO: 12 - protein, 342 aa, Candida sp.
MKLLSLTGVAGVLATCVAATPLVKRLPSGSDPAFSQPKSVLDAGLTCQGASPSSVSKPILLVPGTGTTGPQSFDSNWIPLSTQLGYTPCWISPPPFMLNDTQVNTEYMVNAITALYAGSGNNKLPVLTWSQGGLVAQWGLTFFPSIRSKVDRLMAFAPDYKGTVLAGPLDALAVSAPSVWQQTTGSALTTALRNAGGLTQIVPTTNLYSATDEIVQPQVSNSPLDSSYLFNGKNVQAQAVCGPLFVIDHAGSLTSQFSYVVGRSALRSTTGQARSADYGITDCNPLPANDLTPEQKVAAAALLAPAAAAIVAGPKQNCEPDLMPYARPFAVGKRTCSGIVTP